European Patent Application EP 4 588 345 A1, published July 23, 2025. Title: Genetically Modified Non-human Mammals, Preparation Methods Therefor, and Applications Thereof. Applicant: RenGene Biotechnology Co., Ltd. The sequence listing filed with the application follows.

SEQUENCE LISTING (83 sequences)

SEQ ID NO: 1 - RNA, 113 nt, synthetic construct
  source 1..113: mol_type = other RNA
gactctctgaggaccagagagtttaagagctatgctggaaacagcatagcaagtttaaataaggctagtccgttatcaacttgaaaaagtggcaccgagtcggtgcttttttt

SEQ ID NO: 2 - RNA, 113 nt, synthetic construct
  source 1..113: mol_type = other RNA
gatctgcatgtgcccattccgtttaagagctatgctggaaacagcatagcaagtttaaataaggctagtccgttatcaacttgaaaaagtggcaccgagtcggtgcttttttt

SEQ ID NO: 3 - RNA, 114 nt, synthetic construct
  source 1..114: mol_type = other RNA
gtccagtgagcagttaacatcgtttaagagctatgctggaaacagcatagcaagtttaaataaggctagtccgttatcaacttgaaaaagtggcaccgagtcggtgcttttttt

SEQ ID NO: 4 - RNA, 113 nt, synthetic construct
  source 1..113: mol_type = other RNA
ggccactgtcacaccactcggtttaagagctatgctggaaacagcatagcaagtttaaataaggctagtccgttatcaacttgaaaaagtggcaccgagtcggtgcttttttt

SEQ ID NO: 5 - RNA, 113 nt, synthetic construct
  source 1..113: mol_type = other RNA
acgatcactgatttctacccgtttaagagctatgctggaaacagcatagcaagtttaaataaggctagtccgttatcaacttgaaaaagtggcaccgagtcggtgcttttttt

SEQ ID NO: 6 - RNA, 113 nt, synthetic construct
  source 1..113: mol_type = other RNA
gctctggtaaagaacgttaggtttaagagctatgctggaaacagcatagcaagtttaaataaggctagtccgttatcaacttgaaaaagtggcaccgagtcggtgcttttttt

SEQ ID NO: 7 - DNA, 23 bp, synthetic construct
  source 1..23: mol_type = other DNA
gactctctgaggaccagagaggg

SEQ ID NO: 8 - DNA, 23 bp, synthetic construct
  source 1..23: mol_type = other DNA
gatctgcatgtgcccattccagg

SEQ ID NO: 9 - DNA, 25 bp, synthetic construct
  source 1..25: mol_type = other DNA
ctgaagggccagatccacctactct

SEQ ID NO: 10 - DNA, 25 bp, synthetic construct
  source 1..25: mol_type = other DNA
ttggggtgtggatcctttgttctcg

SEQ ID NO: 11 - DNA, 23 bp, synthetic construct
  source 1..23: mol_type = other DNA
tccagtgagcagttaacatctgg

SEQ ID NO: 12 - DNA, 25 bp, synthetic construct
  source 1..25: mol_type = other DNA
caagattgtatatatgtgcatcctg

SEQ ID NO: 13 - DNA, 24 bp, synthetic construct
  source 1..24: mol_type = other DNA
cactgccatcaatcttccacttga

SEQ ID NO: 14 - DNA, 23 bp, synthetic construct
  source 1..23: mol_type = other DNA
ggccactgtcacaccactcgggg

SEQ ID NO: 15 - DNA, 23 bp, synthetic construct
  source 1..23: mol_type = other DNA
acgatcactgatttctacccagg

SEQ ID NO: 16 - DNA, 23 bp, synthetic construct
  source 1..23: mol_type = other DNA
ggtgaggaaaaggaaaaagtgcc

SEQ ID NO: 17 - DNA, 25 bp, synthetic construct
  source 1..25: mol_type = other DNA
caaatcccaaagtctggttctgaag

SEQ ID NO: 18 - DNA, 24 bp, synthetic construct
  source 1..24: mol_type = other DNA
gcttgtacccagaaggcatagatt

SEQ ID NO: 19 - DNA, 23 bp, synthetic construct
  source 1..23: mol_type = other DNA
gctctggtaaagaacgttagggg

SEQ ID NO: 20 - DNA, 29 bp, synthetic construct
  source 1..29: mol_type = other DNA
gcagactgtgtgctacagtggagtttcaa

SEQ ID NO: 21 - DNA, 24 bp, synthetic construct
  source 1..24: mol_type = other DNA
caattgtgccagttaaggtgtcag

SEQ ID NO: 22 - DNA, 32 bp, synthetic construct
  source 1..32: mol_type = other DNA
gaaggatataaccaccgtaaacttcccacctg

SEQ ID NO: 23 - DNA, 23 bp, synthetic construct
  source 1..23: mol_type = other DNA
ggtgaggaaaaggaaaaagtgcc

SEQ ID NO: 24 - DNA, 23 bp, synthetic construct
  source 1..23: mol_type = other DNA
tggtaggcaaaagcaccaaggat

SEQ ID NO: 25 - DNA, 24 bp, synthetic construct
  source 1..24: mol_type = other DNA
gcttgtacccagaaggcatagatt

SEQ ID NO: 26 - DNA, 25 bp, synthetic construct
  source 1..25: mol_type = other DNA
tcaccagggagtttgtgctaagctg

SEQ ID NO: 27 - DNA, 25 bp, synthetic construct
  source 1..25: mol_type = other DNA
ggagaagggtcagacgtgaaacctg

SEQ ID NO: 28 - DNA, 25 bp, synthetic construct
  source 1..25: mol_type = other DNA
acaactcaagtgtccatcgactgcc

SEQ ID NO: 29 - DNA, 25 bp, synthetic construct
  source 1..25: mol_type = other DNA
ctcagcacccactgctgttctgtaa

SEQ ID NO: 30 - DNA, 25 bp, synthetic construct
  source 1..25: mol_type = other DNA
ttcccatgtgagccagtttccttcc

SEQ ID NO: 31 - DNA, 25 bp, synthetic construct
  source 1..25: mol_type = other DNA
ggctgcaccgttatttcctctgtct

SEQ ID NO: 32 - DNA, 25 bp, synthetic construct
  source 1..25: mol_type = other DNA
agagggcaaggctcaggaaaagttc

SEQ ID NO: 33 - DNA, 25 bp, synthetic construct
  source 1..25: mol_type = other DNA
accgatttatgacactggtgcaggg

SEQ ID NO: 34 - DNA, 26 bp, synthetic construct
  source 1..26: mol_type = other DNA
ggacactgtacaacccatctgtgctt

SEQ ID NO: 35 - DNA, 26 bp, synthetic construct
  source 1..26: mol_type = other DNA
gacgtggtctattctgttgtcccacc

SEQ ID NO: 36 - DNA, 26 bp, synthetic construct
  source 1..26: mol_type = other DNA
tacattgtgtgagtgacagggcagtg

SEQ ID NO: 37 - DNA, 26 bp, synthetic construct
  source 1..26: mol_type = other DNA
atgaggagatgtgctctcaggggatt

SEQ ID NO: 38 - DNA, 22 bp, synthetic construct
  source 1..22: mol_type = other DNA
ccaaggacactctcatctgccc

SEQ ID NO: 39 - DNA, 24 bp, synthetic construct
  source 1..24: mol_type = other DNA
ccatggttgaggagttttcatctc

SEQ ID NO: 40 - DNA, 23 bp, synthetic construct
  source 1..23: mol_type = other DNA
gggaatgcaaatctccaccagct

SEQ ID NO: 41 - DNA, 24 bp, synthetic construct
  source 1..24: mol_type = other DNA
caaacaggactcagcttctgcttc

SEQ ID NO: 42 - DNA, 24 bp, synthetic construct
  source 1..24: mol_type = other DNA
gcagtcaccagagctccagacaat

SEQ ID NO: 43 - DNA, 27 bp, synthetic construct
  source 1..27: mol_type = other DNA
cagtttaagacacagcaagaagttcca

SEQ ID NO: 44 - DNA, 25 bp, synthetic construct
  source 1..25: mol_type = other DNA
cactgaaagaaatcggcctccagtg

SEQ ID NO: 45 - DNA, 25 bp, synthetic construct
  source 1..25: mol_type = other DNA
gtggggtgatgtcttggggagagtc

SEQ ID NO: 46 - DNA, 25 bp, synthetic construct
  source 1..25: mol_type = other DNA
ttcatgcccctagagttggctgaag

SEQ ID NO: 47 - DNA, 25 bp, synthetic construct
  source 1..25: mol_type = other DNA
tggagtggagctctggtctagtgac

SEQ ID NO: 48 - DNA, 27 bp, synthetic construct
  source 1..27: mol_type = other DNA
atgaaatgcagctggggcatsttcttc

SEQ ID NO: 49 - DNA, 26 bp, synthetic construct
  source 1..26: mol_type = other DNA
atgggatggagctrtatcatsytctt

SEQ ID NO: 50 - DNA, 27 bp, synthetic construct
  source 1..27: mol_type = other DNA
atgaagwtgtggttaaactgggttttt

SEQ ID NO: 51 - DNA, 25 bp, synthetic construct
  source 1..25: mol_type = other DNA
atgractttgggytcagcttgrttt

SEQ ID NO: 52 - DNA, 32 bp, synthetic construct
  source 1..32: mol_type = other DNA
atgggactccaggcttcaatttagttttcctt

SEQ ID NO: 53 - DNA, 29 bp, synthetic construct
  source 1..29: mol_type = other DNA
atggcttgtcyttrgsgctrctcttctgc

SEQ ID NO: 54 - DNA, 27 bp, synthetic construct
  source 1..27: mol_type = other DNA
atggratggagckggrgtctttmtctt

SEQ ID NO: 55 - DNA, 23 bp, synthetic construct
  source 1..23: mol_type = other DNA
atgagagtgctgattcttttgtg

SEQ ID NO: 56 - DNA, 31 bp, synthetic construct
  source 1..31: mol_type = other DNA
atggmttgggtgtggamcttgcttattcctg

SEQ ID NO: 57 - DNA, 28 bp, synthetic construct
  source 1..28: mol_type = other DNA
atgggcagacttaccattctcattcctg

SEQ ID NO: 58 - DNA, 28 bp, synthetic construct
  source 1..28: mol_type = other DNA
atggattttgggctgattttttttattg

SEQ ID NO: 59 - DNA, 26 bp, synthetic construct
  source 1..26: mol_type = other DNA
atgatggtgttaagtccttctgtacc

SEQ ID NO: 60 - DNA, 18 bp, synthetic construct
  source 1..18: mol_type = other DNA
gttcatctctgcgacagc

SEQ ID NO: 61 - DNA, 20 bp, synthetic construct
  source 1..20: mol_type = other DNA
ctgcatccttcccagtggag

SEQ ID NO: 62 - DNA, 18 bp, synthetic construct
  source 1..18: mol_type = other DNA
gaggtgcagctggtgcag

SEQ ID NO: 63 - DNA, 18 bp, synthetic construct
  source 1..18: mol_type = other DNA
gaggtgcagctggtggag

SEQ ID NO: 64 - DNA, 18 bp, synthetic construct
  source 1..18: mol_type = other DNA
gaggtgcagctgttggag

SEQ ID NO: 65 - DNA, 18 bp, synthetic construct
  source 1..18: mol_type = other DNA
caggtgcagctgcaggag

SEQ ID NO: 66 - DNA, 20 bp, synthetic construct
  source 1..20: mol_type = other DNA
caggtgcagctacagcagtg

SEQ ID NO: 67 - DNA, 18 bp, synthetic construct
  source 1..18: mol_type = other DNA
caggttcagctggtgcag

SEQ ID NO: 68 - DNA, 18 bp, synthetic construct
  source 1..18: mol_type = other DNA
caggtccagctggtacag

SEQ ID NO: 69 - DNA, 18 bp, synthetic construct
  source 1..18: mol_type = other DNA
gaagtgcagctggtggag

SEQ ID NO: 70 - DNA, 18 bp, synthetic construct
  source 1..18: mol_type = other DNA
caggtacagctgcagcag

SEQ ID NO: 71 - DNA, 18 bp, synthetic construct
  source 1..18: mol_type = other DNA
cagctgcagctgcaggag

SEQ ID NO: 72 - DNA, 18 bp, synthetic construct
  source 1..18: mol_type = other DNA
tgaggagacggtgaccag

SEQ ID NO: 73 - DNA, 20 bp, synthetic construct
  source 1..20: mol_type = other DNA
tgaagagacggtgaccattg

SEQ ID NO: 74 - DNA, 19 bp, synthetic construct
  source 1..19: mol_type = other DNA
tgaggagacggtgaccgtg

SEQ ID NO: 75 - protein, 11 aa, unidentified
GPPPPCPPCPP

SEQ ID NO: 76 - DNA, 9125 bp, synthetic construct
  source 1..9125: mol_type = other DNA
agcacgattgaagtgctgattcaaaggctgcacacatataccaacattttccatatcgtacactataaatttgaattcactattgattgaatttttgaataaagcagtaacaaaaatgagtatattggctgaggaagagcaagaaagagatgaatattgacacttgaataatcacggactcctgaaaatacacacatgtgaacactgattgcatatttcaggtaaatactagaaaaagcaaagtcacataaagtcgttatgacaggtgggataccctgcaaatcacactaggcatgtcccacactgccctggagctgtctcaggggagcagtctcctccagtgtttagaggcacaggcacggataatagggctgacgctgtccagatgtgtgatattggacacattgcacaactgctctgttatgtatgtaattcatcttctctaaaaatgtaacattgacacttgcactgaatatattctgcaaatatgtaaacattaaataagatgatgactgctaattgatcatcaagtcacaatcacataatctgaagttatattttcctgagagataggattacctccagtgttttccgggaccctctcatctgctctgggcactgccctctcctccagcgtcccactagagcttgctatatagtaggagacatgcaaatagggccctccctctgctgataaaaaccagccgagcccagaccctgcagctctgggagaagagccccagccccagaattcccaggagtttccattcggtgatcagcactgaacacagaggactcaccatggagtttgggctgagctgggttttccttgttgctattataaaaggtgatttatggagaactagagacattgagtggacgtgagtgagataagcagtgaatatatgtggcagtttctgaccaggttgtctctgtgtttgcaggtgtccagtgtcaggtgcagctggtggagtctgggggaggcttggtcaagcctggagggtccctgagactctcctgtgcagcctctggattcaccttcagtgactactacatgagctggatccgccaggctccagggaaggggctggagtgggtttcatacattagtagtagtagtagttacacaaactacgcagactctgtgaagggccgattcaccatctccagagacaacgccaagaactcactgtatctgcaaatgaacagcctgagagccgaggacacggctgtgtattactgtgcgagagacacagtgaggggaggtcagtgtgagcccagacacaaacctccctgcaggggtccccaggaccaccagggggcgcccgggacactgtgcacggggctgtctccagggcaggtgcaggtgctgctgagggctggcttcctgtcatggcctggggctgcctcattgtcaaatttccccaggaacttctccagatttacaattctgtactaacatttgatgtctctaaatgcaatactttttttgtcctttttgtttctttgtttttttgcaacaggagtacatatcctcagctccacagaagccagggtgtcactttgggggcagaaataatcctttcatggttaccaggataagagtcctgaggaatcccagggaaacctggagagtgttttccagttagactcagggcagagacctccatgggaatctctgattagaacaggccttgagctctgacgggagccaagagagaggctcgcccagggtcagagtccttaaaacctgatggttttcacagctatcccccctcgtcttgtaaactcagactgattcagttgaccctctttctgctaatccatttccttctctgtaggtttgattctcacagttcgctttcttcttctcttccctgaaaacagacgatgtgttttctgtagtcaaaatcccagggctcaggtctgcaggacctgggtaggctacggggactttctcactcaccattgtccggacactcttgtcttctgtgcatggaggcatttggaaaatgaagtggacattagccatgaagggaataatactagttttctccaataggatattgatgtagagctgatcttgtgcttctcacactgtctcagagtttggactctcacctgtgactttgagaagagctggggatgggcactccattgtgctgtgagctctgggtaacgataattgtagaatctgcctaggcagtctaaggtcaatactactcgtcatcaggaaagacagctggaattcctgggaagatctgcatctgccgtccaccatggagtcccatcgtcttctgttatgctctctttgaatcagtcccacctagattatctagaacactcttcctgacttaggaaaaataatggcaggctccactaacacctgtgttatgccatgggagcaacacctaagctagtgtgtgaatgagtagatgagactgtggtctagtcaaggtgacaggtaaaattgattgttgccattatgatattttattttatatttggcaatatagtcatgctcctattataaatattctttgagacggagtcttgctctgttgccagcctggagagtgcagcagcacgatctcggctcactgcaacctcttccacctcccaggttcaagcagttctcctgcctcagcctcccgagaaactgggattacaggtgcacgccaccatgcctggctaatttttgtatttttagtatcgacagggtttcaccatgtgggccagtgtggtctcgatttcctgacctcgtgatctgcacacctcggcctcccaaagtgctgggattacaggcatgagccaccacacctggcctagttttattaatgtctgcccataccagcaactacatacctatggggacattaatttacatctgcagacatatgtgtaaatacacaagcctatacatacatgtgtagccatttatatttaacattataataaaataattctaaaatattttctaaagaattaaacttaatgatgagctaaatataaattagagtaatctataattgatttcgatcattctctatagtttgcataaatggatgtctatttctaagccttaacatagtgtattcgtcattttaaaatagtcaagaaaaaattacaaatgttcttgtcacaaaaaaagataaggatttgatgatttgaggtaatatatatgtcaattaactcgattcaattattccgtattgcattcacaaaccataacatacctttgtgccccataaatatatacaaccaaaatttctcaattttcaatgaaattttaattatatatttttaaatctgatgcctctccttggattaagccacctcctcaggcttacagggctcttccattttctcaacatgttgttataccagatgagcacaaacacattaatttcattatgcttagctttaatttttcaaaacaacataaaggtgataattttaccaatagacgtattacaacctactgtgcatgagaccctttctgtgcttcaaggtttcttctcaggactttatatgtattgcaaattttcatttttttctgatatggaatgctgatttctctttattatagattatcagtttatttttcaaatttatctcttaaaattaattttttcaaagtcccactcaaaccagggtattattagaactttgacgtgtaatagttggaccaactttgagaatacattcaatttagttcacgtgctctcaagcatcttttcttctttaaaagttgttgtcagttgtaatatcacacaaaatattagtaatttatgctaatgacaggttaaaatgctgtataaataattaaattacatttgattggaaaaaaggaatagatgttcctcatatcttgactttttttcttctctatgagatgcatgcttattaattattaagtttaagacgttacccttgtctttttgatttctgggatttaattttagtacatatacttgaatgcattgtattaattcatataataatgttcatattttggatagggttttaatattaattttattattactgaattttaaactattctacactttttttgtttttatgagataaaatttacatataagaaaatatgcatagatctggaatgtatcactagagagtttctggcaaatgtgaatacccttgttgtccccagcacctaaggtagctgaagagcaagtccattcccacatcgcgggtctttccctgtgcctgaggtcagctcctgcatggggaaatgttttgatttctcacactacagatccatttttttctgttttgaactttatataaatggaatcaaacattatagacctttttttggaaaggagctttgctatttttgagattaattcatgctatttaatgtgtaaaattagatcaacatattgtcatttatttaattcatggactgactctgatatgaaacctcaaagttttcatgtatatatggagacagggagaggaaggagaaagattttatatctgagtcagtccattaagtaaataaatgagaatattttgatttattttcttgtcgatgtactttaaatttgtttccattttatgaatattataggcaaagctgttacaaatatattagtgtaggttttcctatgttgtctcatttttattgagaaaatatgaagtatgtatttctttatttttttatttttgattattatttatttatattttaaattttactttaagttctgggatacatgtgctgaacgtgcaggtttgttacataagtatacatgtgccgtggcggtttgctgcacatatcaaccagtcatctatgtttgaagcgcctcaggcattaggtatttgtcctaatgctctccctcccccttcctcccacccctgatgcatcctagtgtgtgacgttcccctccctgtgtccatgtgttctcattgttcaactcccacttttgagtgaaaacatgcggtgtttggttttctgttcctgtgttagtttgttgaggatgatgatttccagcttcatccatgtccctgcaaaggacatgacatcattcttttttgtggctgcatagaattccatggtgtatatatgccacattttctttatccagtctatcattgatggttatcacatggttatcacattctttggttttcatttaggagcatatgtcttgagtagaaatttggtcctttccacacactaagcctcaccttcctcagaggaagagcagagattcatccaactttgtctgaggtgggagctgcttctccacaccttggagcttgcagagacccctaagtgcagcttcattgagtcaggtgtgtctccatgtgggggacttctgctgccagtgattgctgctcagttctaattgtgggttcggaattaggacacttaggttatcacgcctcaaaaattaccatcattatagagaaaaataataatacaatgctaatcattgtcacttattacttattattattggagtataagtttggagagacaaaattgttaccatatatttgcataaatgtaatgtcagaatctcctgaatgggtcttgaacacttacaaactggatagaagcagattcttattttttttctatactggtgtattttgggatgtcaacattttgtccagaatctgtgagtaccaataactgtgtgtttcaagactcttcttgggttctgagacaagaaatgccattactacctgaaggattgagacaactttgaacaatgtcagagcaatcatctctaattgcttctaaacttcagttttatcaattcttatgctctctgaattatttctgattttagctattaaaggattctctctttttctcttagttaattgagctaagaatttgtctatttttttagaaaaaatctctttgatttgttgatttttctattgcttgtaaagtccatttttcacttacttatttcatttactctaaagcctcataaacacattggtgacatgtagatagagaatttgatcgtaaatgccatgtttttgttagactcagctgatcatgtcaggaagccccctgagggttctaggaactgactgtggctcccaccactggacaaggatgagaacctccatgctttggggatgggaggacatgcagggcagtgtgaggggaggagggttgctggcaggtccagcattgcttcccctggctgcaccactcatgtccttcctcactcagagattcagtcatttcttcccaggtggaaaaatcagttaactttatctttgatatatggatgggagcccaagatagaggcttgtcagtcattatttctgtgcctgctgccttgggaatgtctgaatttcttatgctctgtcctgggtctataccccagtggctcccctactccatggcacccacctgtgcctgtgcatggcccctgatcacagcctccgtgaaacatctggtttggctcaggaagaaccccccttgccttgttttcctgctgtccctggtccacatccttctccatccacaggctctcagtggtgcctcccatccacactgaccctacatggggtcataccttgtccaccacttcctctctctttctcgagctgcggccgctttcacgtagaaagccagtccgcagaaacggtgctgaccccggatgaatgtcagctactgggctatctggacaagggaaaacgcaagcgcaaagagaaagcaggtagcttgcagtgggcttacatggcgatagctagactgggcggttttatggacagcaagcgaaccggaattgccagctggggcgccctctggtaaggttgggaagccctgcaaagtaaactggatggctttcttgccgccaaggatctgatggcgcaggggatcaagctctgatcaagagacaggatgaggatcgtttcgcatgattgaacaagatggattgcacgcaggttctccggccgcttgggtggagaggctattcggctatgactgggcacaacagacaatcggctgctctgatgccgccgtgttccggctgtcagcgcaggggcgcccggttctttttgtcaagaccgacctgtccggtgccctgaatgaactgcaagacgaggcagcgcggctatcgtggctggccacgacgggcgttccttgcgcagctgtgctcgacgttgtcactgaagcgggaagggactggctgctattgggcgaagtgccggggcaggatctcctgtcatctcaccttgctcctgccgagaaagtatccatcatggctgatgcaatgcggcggctgcatacgcttgatccggctacctgcccattcgaccaccaagcgaaacatcgcatcgagcgagcacgtactcggatggaagccggtcttgtcgatcaggatgatctggacgaagagcatcaggggctcgcgccagccgaactgttcgccaggctcaaggcgagcatgcccgacggcgaggatctcgtcgtgacccatggcgatgcctgcttgccgaatatcatggtggaaaatggccgcttttctggattcatcgactgtggccggctgggtgtggcggaccgctatcaggacatagcgttggctacccgtgatattgctgaagagcttggcggcgaatgggctgaccgcttcctcgtgctttacggtatcgccgctcccgattcgcagcgcatcgccttctatcgccttcttgacgagttcttctgatgtacatttctccttacgcatctgtgcggtatttcacaccgcatatggtgcactctcagtacaatctgctctgatgccgcatagttaagccagccccgacacccgccaacacccgctgacgcgaaccccttgcggccgcatcgaatataacttcgtataatgtatgctatacgaagttattagcgatgagctcggacttccattgttcattccacggacaaaaacagagaaaggaaacgacagaggccaaaaagctcgctttcagcacctgtcgtttcctttcttttcagagggtattttaaataaaaacattaagttatgacgaagaagaacggaaacgccttaaaccggaaaattttcataaatagcgaaaacccgcgaggtcgccgccccgtaacctgtcggatcaccggaaaggacccgtaaagtgataatgattatcatctacatatcacaacgtgcgtggaggccatcaaaccacgtcaaataatcaattatgacgcaggtatcgtattaattgatctgcatcaacttaacgtaaaaacaacttcagacaatacaaatcagcgacactgaatacggggcaacctcatgtccgagctcgcgagctcgtcgacagcgacacacttgcatcggatgcagcccggttaacgtgccggcacggcctgggtaaccaggtattttgtccacataaccgtgcgcaaaatgttgtggataagcaggacacagcagcaatccacagcaggcatacaaccgcacaccgaggttactccgttctacaggttacgacgacatgtcaatacttgcccttgacaggcattgatggaatcgtagtctcacgctgatagtctgatcgacaatacaagtgggaccgtggtcccagaccgataatcagaccgacaacacgagtgggatcgtggtcccagactaataatcagaccgacgatacgagtgggaccgtggtcccagactaataatcagaccgacgatacgagtgggaccgtggttccagactaataatcagaccgacgatacgagtgggaccgtggtcccagactaataatcagaccgacgatacgagtgggaccatggtcccagactaataatcagaccgacgatacgagtgggaccgtggtcccagtctgattatcagaccgacgatacgagtgggaccgtggtcccagactaataatcagaccgacgatacgagtgggaccgtggtcccagactaataatcagaccgacgatacgagtgggaccgtggtcccagtctgattatcagaccgacgatacaagtggaacagtgggcccagagagaatattcaggccagttatgctttctggcctgtaacaaaggacattaagtaaagacagataaacgtagactaaaacgtggtcgcatcaggg

SEQ ID NO: 77 - DNA, 8890 bp, synthetic construct
  source 1..8890: mol_type = other DNA
ggcccgtttttggactcctgggggtgacttagcagccgtctgcttgcagttggacttcccaggccgacagtggtctggcttctgaggggtcaggccagaatgtggggtacgtgggaggccagcagagggttccatgagaagggcaggacagggccacggacagtcagcttccatgtgacgcccggagacagaaggtctctgggtggctgggtttttgtggggtgaggatggacattctgccattgtgattactactactactactacatggacgtctggggcaaagggaccacggtcaccgtctcctcaggtaagaatggccactctagggcctttgttttctgctactgcctgtggggtttcctgagcattgcaggttggtcctcggggcatgttccgaggggacctgggcggactggccaggaggggacgggcactggggtgccttgaggatctgggagcctctgtggattttccgatgcctttggaaaatgggactcaggttgggtgcgtctgatggagtaactgagcctgggggcttggggagccacatttggacgagatgcctgaacaaaccaggggtcttagtgatggctgaggaatgtgtctcaggagcggtgtctgtaggactgcaagatcgctgcacagcagcgaatcgtgaaatattttctttagaattatgaggtgcgctgtgtgtcaacctgcatcttaaattctttattggctggaaagagaactgtcggagtgggtgaatccagccaggagggacgcgtagccccggtcttgatgagagcagggttgggggcaggggtagcccagaaacagtggctgccgtcctgacaggggcttagggaggctccaggacctcagtgccttgaagctggtttccatgagaaaaggattgtttatcttaggaggcatgcttactgttaaaagacagggtcctatggctggagggatagttggggctgtagttggagattttcagtttttagaataaaagtattagttgtggaatatacttcaggaccacctctgtgacagcatttatacagtatccgatgcatagggacaaagagtggagtggggcactttctttagatttgtgaggaatgttccgcactagattgtttaaaacttcatttgttggaaggagagctgtcttagtgattgagtcaagggagaaaggcatctagcctcggtctcaaaagggtagttgctgtctagagaggtctggtggagcctgcaaaagtccagctttcaaaggaacacagaagtatgtgtatggaatattagaagatgttgcttttactcttaagttggttcctaggaaaaatagttaaatactgtgactttaaaatgtgagagggttttcaagtactcatttttttaaatgtccaaaattcttgtcaatcagtttgaggtcttgtttgtgtagaactgatattacttaaagtttaaccgaggaatgggagtgaggctctctcataacctattcagaactgacttttaacaataataaattaagtttcaaatatttttaaatgaattgagcaatgttgagttggagtcaagatggccgatcagaaccagaacacctgcagcagctggcaggaagcaggtcatgtggcaaggctatttggggaagggaaaataaaaccactaggtaaacttgtagctgtggtttgaagaagtggttttgaaacactctgtccagccccaccaaaccgaaagtccaggctgagcaaaacaccacctgggtaatttgcatttctaaaataagttgaggattcagccgaaactggagaggtcctcttttaacttattgagttcaaccttttaattttagcttgagtagttctagtttccccaaacttaagtttatcgacttctaaaatgtatttagaattcattttcaaaattaggttatgtaagaaattgaaggactttagtgtctttaatttctaatatatttagaaaacttcttaaaattactctattattcttccctctgattattggtctccattcaattcttttccaatacccgaagcatttacagtgactttgttcatgatcttttttagttgtttgttttgccttactattaagactttgacattctggtcaaaacggcttcacaaatctttttcaagaccactttctgagtattcattttaggagaaagactttttttttaaatgaatgcaattatctagacttatttcagttgaacatgctggttggtggttgagaggacactcagtcagtcagtgacgtgaagggcttctaagccagtccacatgctctgtgtgaactccctctggccctgcttattgttgaatgggccaaaggtctgagaccaggctgctgctgggtaggcctggactttgggtctcccacccagacctgggaatgtatggttgtggcttctgccacccatccacctggctgctcatggaccagccagcctcggtggctttgaaggaacaattccacacaaagactctggacctctccgaaaccaggcaccgcaaatggtaagccagaggcagccacagctgtggctgctgctcttaaagcttgtaaactgtttctgcttaagagggactgagtcttcagtcattgctttagggggagaaagagacatttgtgtgtcttttgagtaccgttgtctgggtcactcacatttaactttccttgaaaaactagtaaaagaaaaatgttgcctgttaaccaataatcatagagctcatggtactttgaggaaatcttagaaagcgtgtatacaattgtctggaattatttcagttaagtgtattagttgaggtactgatgctgtctctacttcagttatacatgtgggtttgaattttgaatctattctggctcttcttaagcagaaaatttagataaaatggatacctcagtggtttttaatggtgggtttaatatagaaggaatttaaattggaagctaatttagaatcagtaaggagggacccaggctaagaaggcaatcctgggattctggaagaaaagatgtttttagtttttatagaaaacactactacattcttgatctacaactcaatgtggtttaatgaatttgaagttgccagtaaatgtacttcctggttgttaaagaatggtatcaaaggacagtgcttagatccgaggtgagtgtgagaggacaggggctggggtatggatacgcagaaggaaggccacagctgtacagaattgagaaagaatagagacctgcagttgaggccagcaggtcggctggactaactctccagccacagtaatgacccagacagagaaagccagactcataaagcttgctgagcaaaattaagggaacaaggttgagagccctagtaagcgaggctctaaaaagcacagctgagctgagatgggtgggcttctctgagtgcttctaaaatgcgctaaactgaggtgattactctgaggtaagcaaagctgggcttgagccaaaatgaagtagactgtaatgaactggaatgagctgggccgctaagctaaactaggctggcttaaccgagatgagccaaactggaatgaacttcattaatctaggttgaatagagctaaactctactgcctacactggactgttctgagctgagatgagctggggtgagctcagctatgctacgctgtgttggggtgagctgatctgaaatgagatactctggagtagctgagatggggtgagatggggtgagctgagctgggctgagctagactgagctgagctagggtgagctgagctgggtgagctgagctaagctggggtgagctgagctgagcttggctgagctagggtgagctgggctgagctggggtgagctgagctgagctggggtaagctgggatgagctggggtgagctgagctgagctggagtgagctgagctgggctgagctggggtgagctgggctgagctgggctgagctgggctgagctggggtgagctgagctggggtgagctgagctgagctggggtgagctgagctgagctggggtgagctggggtgagctgagctggggtgagctgagctgagctggggtgagctgagctggggtgagctgagctgagctggggtgagctgagctgagctgagctgagctgagctggggtgagctgagctgagctgagctggggtgagctggggtgagctgagctgagctggagtgagctgagctgggctgagctggggtgagctgggctgagctggggtgagctgagctgagctgagctgagctggggtgagctgagctgagctggggtgagctgagctggggtgagctgggctgagctgagctgagctgagctgagctgagctgagctgagctgagctgagctgagctgagctgagctgagctgagctgagctgagctggggtgagctgagctgagctgggctgagctggggtgagctgggctgagctgggctgagctgggctgagctggggtgagctgagctggggtgagctgagctgagctgggctgagctgagctgagctggggtgagctgagctgagctggggtgagctgagctgagctgagctggggtgagctgagctgggctgagcagggctgagctggggtgagctgagctgagctggggtgagctgggctgagctgggctgagctgagctgagctgggctgagctgggctgagctgggctgagctgggctgagctgggctgagctggggtgagctgagctgagctggggtgagctggggtgagctgagctggggtgagctgagctggggtgagctgagctgagctggggtgagctgagctggggtgagctgagctgagctggggtgagctgagctgagctggggtgagctgagctagggtgaactgggctgggtgagctggagtgagctgagctgaggtgaactggggtgagccgggatgttttgagttgagctggggtaagatgagctgaactggggtaaactgggatgagctgtggtgagcggagctggattgaactgagctgtgtgagctgagctggggtcagctgagcaagagtgagtagagctggctggccagaaccagaatcaattaggctaagtgagccagattgtgctgggatcagctgtactcagatgagctgggatgaggtaggctgggatgagctgggctagctgacatggattatgtgaggctgagctagcatgggctggcctagctgatgagctaagcttgaatgagcggggctgagctggactcagatgtgctagactgagctgtactggatgatctggtgtagggtgatctggactcaactgggctggctgatgggatgcgccaggttgaactaggctcagataagttaggctgagtagggcctggttgagatggttcgggatgagctgggaaaagatggactcggaccatgaactgggctgagctgggttgggagaccatgaattgagctgaactgagtgcagctgggataaactgggttgagctaagaatagactacctgaattgtgccaaactcggctgggatcaattggaaattatcaggatttagatgagccggactaaactatgctgagctggactggttggatgtgttgaactggcctgctgctgggctggcatagctgagttgaacttaaatgaggaaggctgagcaaggctagcctgcttgcatagagctgaactttagcctagcctgagctggaccagcctgagctgagtaggtctaaactgagttaaaaatcaacagggataatttaacagctaatttaacaagcctgaggtctgagattgaatgagcagagctgggatgaactgaatgagtttcaccaggcctggaccagttaggctaggacctcgttctatagaggcagactgtgtgctacagtggagtttcaagatgattccatgagtcctccccgcccccaacataacccaccttcctcctaccctacacgcctgtctggtgtgtaaatcccagctttgtgtgctgatacagaagcctgagcccctcccccacctccacctacctattactttgggatgagaatagttctcccagccagtgtctcagagggaagccaagcaggacaggcccaaggctacttgagaagccaggatctaggcctctccctgagaacgggtgttcatgcccctagagttggctgaagggccagatccacctactctagaggcatctctccctgtctgtgaaggcttccaaagtcacgttcctgtggctagaaggcagctccatagccctgctgcagtttcgtcctgtataccaggttcacctactaccatatctagccctgcctgccttaagagtagcaacaaggaaatagcagggtgtagagggatctcctgtctgacaggaggcaagaagacagattcttacccctccatttctcttttatccctctctggtcctcagagagtcagtccttcccaaatgtcttccccctcgtccctctgcagaagggccaattcgcggccgctcagaagaactcgtcaagaaggcgatagaaggcgatgcgctgcgaatcgggagcggcgataccgtaaagcacgaggaagcggtcagcccattcgccgccaagctcttcagcaatatcacgggtagccaacgctatgtcctgatagcggtccgccacacccagccggccacagtcgatgaatccagaaaagcggccattttccaccatgatattcggcaagcaggcatcgccatgggtcacgacgagatcctcgccgtcgggcatgctcgccttgagcctggcgaacagttcggctggcgcgagcccctgatgctcttcgtccagatcatcctgatcgacaagaccggcttccatccgagtacgtgctcgctcgatgcgatgtttcgcttggtggtcgaatgggcaggtagccggatcaagcgtatgcagccgccgcattgcatcagccatgatggatactttctcggcaggagcaaggtgagatgacaggagatcctgccccggcacttcgcccaatagcagccagtcccttcccgcttcagtgacaacgtcgagcacagctgcgcaaggaacgcccgtcgtggccagccacgatagccgcgctgcctcgtcttgcagttcattcagggcaccggacaggtcggtcttgacaaaaagaaccgggcgcccctgcgctgacagccggaacacggcggcatcagagcagccgattgtctgttgtgcccagtcatagccgaatagcctctccacccaagcggccggagaacctgcgtgcaatccatcttgttcaatcatgcgaaacgatcctcatcctgtctcttgatcagagcttgatcccctgcgccatcagatccttggcggcaagaaagccatccagtttactttgcagggcttcccaaccttaccagagggcgccccagctggcaattccggttcgcttgctgtccataaaaccgcccagtctagctatcgccatgtaagcccactgcaagctacctgctttctctttgcgcttgcgttttcccttgtccagatagcccagtagctgacattcatccggggtcagcaccgtttctgcggactggctttctacgtgaaagtcgacgcaggtcaccgcgagagtctattttaggaagcaaaaaaacacaattggtaaatttatcacttctggttgtgaagaggtggttttgcccaggcccagatctgaaagtgctctactgagcaaaacaacacctggacaatttgcgtttctaaaataaggcgaggctgaccgaaactgaaaaggctttttttaactatctgaatttcatttccaatcttagcttatcaactgctagtttgtgcaaacagcatatcaacttctaaactgcattcatttttaaagtaagatgtttaagaaattaaacagtcttagggagagtttatgactgtattcaaaaagttttttaaattagcttgttatcccttcatgtgataattaatctcaaatactttttcgatacctcagagcattattttcataatgactgtgttcacaatctttttaggttaactcgttttctctttgtgattaaggagaaacactttgatattctgatagagtggccttcattttagtatttttcaagaccacttttcaactactcactttaggataagttttaggtaaaatgtgcatcattatcctgaattatttcagttaagcatgttagttggtggcataagagaaaactcaatcagatagtgctgaagacaggactgtggagacaccttagaaggacagattctgttccgaatcaccgatgcggcgtcagcaggactggcctagcggaggctctgggagggtggctgccaggcccggcctgggctttgggtctccccggactacccagagctgggatgcgtggcttctgctgccgggccgactggctgctcaggccccagcccttgttaatggacttggaggaatgattccatgccaaagctttgcaaggctcgcagtgaccaggcgcccgacatggtaagagacaggcagccgccgctgctgcatttgcttctcttaaaactttgtatttgacgtcttatttccactagaaggggaactggtcttaattgcttgatgaagagcaggagactcatttatgtgagtcttttgagtgaccattgtctgggtcactcccatttaactttccctaaagcccatttgaaggagaggtcgcacgagctgctccacaacctctgaatggggatggcatgggtaatgatgcttgagaacataccaagccccactggcatcgcccttgtctaagtcattgactgtaggtcatcatcgcacccttgaaagtagcccatgccatcgatg

SEQ ID NO: 78 - DNA, 8000 bp, synthetic construct
  source 1..8000: mol_type = other DNA
ccaagccatggaggagaagagcttgactctggtgtgagttcaattcagactgcttctgaatatgatctttgacaagtatggtgaccaggagatggaatgtgagcctccaccatgaaggatcactacctgaatgaaagtagcatagacagactccagaaggcagattaaacaggaaatcctatcaacttgaactaagttaccttttctggttatgtctgcccaacctgatttgtctaggcaggaggctggtccagcttgacatccaatggaatggactcctcagttccaacgccattctcccaccagttttcttgtccacttggtcttgctggccaagtagactacattgcagatgaaggtcttgttagtccaggtgctggcaggattagtcactgagccactaaggaaatagaatccagactgcagaacatgtaggaagatgtacacaccactgcacagggaacaggggttccaggacataatcatttgttcaggtacaccactagacaaggctccaggattccagtatacatgtccatcagctcaagaaactagcctttatccaggcatccccagatcaccatggagccagaaatgtccccacagccaggatctagaaagaaaacatgggactgtggttctggctacaagataggggggatatgtgagtatcctatcagacatatctgggtctaagacatctttctaatccttcccagggcgctggccctttgcaaactcgaggcggccgctcagaagaactcgtcaagaaggcgatagaaggcgatgcgctgcgaatcgggagcggcgataccgtaaagcacgaggaagcggtcagcccattcgccgccaagctcttcagcaatatcacgggtagccaacgctatgtcctgatagcggtccgccacacccagccggccacagtcgatgaatccagaaaagcggccattttccaccatgatattcggcaagcaggcatcgccatgggtcacgacgagatcctcgccgtcgggcatgctcgccttgagcctggcgaacagttcggctggcgcgagcccctgatgctcttcgtccagatcatcctgatcgacaagaccggcttccatccgagtacgtgctcgctcgatgcgatgtttcgcttggtggtcgaatgggcaggtagccggatcaagcgtatgcagccgccgcattgcatcagccatgatggatactttctcggcaggagcaaggtgagatgacaggagatcctgccccggcacttcgcccaatagcagccagtcccttcccgcttcagtgacaacgtcgagcacagctgcgcaaggaacgcccgtcgtggccagccacgatagccgcgctgcctcgtcttgcagttcattcagggcaccggacaggtcggtcttgacaaaaagaaccgggcgcccctgcgctgacagccggaacacggcggcatcagagcagccgattgtctgttgtgcccagtcatagccgaatagcctctccacccaagcggccggagaacctgcgtgcaatccatcttgttcaatcatgcgaaacgatcctcatcctgtctcttgatcagagcttgatcccctgcgccatcagatccttggcggcaagaaagccatccagtttactttgcagggcttcccaaccttaccagagggcgccccagctggcaattccggttcgcttgctgtccataaaaccgcccagtctagctatcgccatgtaagcccactgcaagctacctgctttctctttgcgcttgcgttttcccttgtccagatagcccagtagctgacattcatccggggtcagcaccgtttctgcggactggctttctacgtgaaagtcgacgcggccgctcctatggctggagggatagttggggctgtagttggagattttcagtttttagaataaaagtattagttgtggaatatacttcaggaccacctctgtgacagcatttatacagtatccgatgcatagggacaaagagtggagtggggcactttctttagatttgtgaggaatgttccgcactagattgtttaaaacttcatttgttggaaggagagctgtcttagtgattgagtcaagggagaaaggcatctagcctcggtctcaaaagggtagttgctgtctagagaggtctggtggagcctgcaaaagtccagctttcaaaggaacacagaagtatgtgtatggaatattagaagatgttgcttttactcttaagttggttcctaggaaaaatagttaaatactgtgactttaaaatgtgagagggttttcaagtactcatttttttaaatgtccaaaattcttgtcaatcagtttgaggtcttgtttgtgtagaactgatattacttaaagtttaaccgaggaatgggagtgaggctctctcataacctattcagaactgacttttaacaataataaattaagtttcaaatatttttaaatgaattgagcaatgttgagttggagtcaagatggccgatcagaaccagaacacctgcagcagctggcaggaagcaggtcatgtggcaaggctatttggggaagggaaaataaaaccactaggtaaacttgtagctgtggtttgaagaagtggttttgaaacactctgtccagccccaccaaaccgaaagtccaggctgagcaaaacaccacctgggtaatttgcatttctaaaataagttgaggattcagccgaaactggagaggtcctcttttaacttattgagttcaaccttttaattttagcttgagtagttctagtttccccaaacttaagtttatcgacttctaaaatgtatttagaattcattttcaaaattaggttatgtaagaaattgaaggactttagtgtctttaatttctaatatatttagaaaacttcttaaaattactctattattcttccctctgattattggtctccattcaattcttttccaatacccgaagcatttacagtgactttgttcatgatcttttttagttgtttgttttgccttactattaagactttgacattctggtcaaaacggcttcacaaatctttttcaagaccactttctgagtattcattttaggagaaagactttttttttaaatgaatgcaattatctagacttatttcagttgaacatgctggttggtggttgagaggacactcagtcagtcagtgacgtgaagggcttctaagccagtccacatgctctgtgtgaactccctctggccctgcttattgttgaatgggccaaaggtctgagaccaggctgctgctgggtaggcctggactttgggtctcccacccagacctgggaatgtatggttgtggcttctgccacccatccacctggctgctcatggaccagccagcctcggtggctttgaaggaacaattccacacaaagactctggacctctccgaaaccaggcaccgcaaatggtaagccagaggcagccacagctgtggctgctgctcttaaagcttgtaaactgtttctgcttaagagggactgagtcttcagtcattgctttagggggagaaagagacatttgtgtgtcttttgagtaccgttgtctgggtcactcacatttaactttccttgaaaaactagtaaaagaaaaatgttgcctgttaaccaataatcatagagctcatggtactttgaggaaatcttagaaagcgtgtatacaattgtctggaattatttcagttaagtgtattagttgaggtactgatgctgtctctacttcagttatacatgtgggtttgaattttgaatctattctggctcttcttaagcagaaaatttagataaaatggatacctcagtggtttttaatggtgggtttaatatagaaggaatttaaattggaagctaatttagaatcagtaaggagggacccaggctaagaaggcaatcctgggattctggaagaaaagatgtttttagtttttatagaaaacactactacattcttgatctacaactcaatgtggtttaatgaatttgaagttgccagtaaatgtacttcctggttgttaaagaatggtatcaaaggacagtgcttagatccgaggtgagtgtgagaggacaggggctggggtatggatacgcagaaggaaggccacagctgtacagaattgagaaagaatagagacctgcagttgaggccagcaggtcggctggactaactctccagccacagtaatgacccagacagagaaagccagactcataaagcttgctgagcaaaattaagggaacaaggttgagagccctagtaagcgaggctctaaaaagcacagctgagctgagatgggtgggcttctctgagtgcttctaaaatgcgctaaactgaggtgattactctgaggtaagcaaagctgggcttgagccaaaatgaagtagactgtaatgaactggaatgagctgggccgctaagctaaactaggctggcttaaccgagatgagccaaactggaatgaacttcattaatctaggttgaatagagctaaactctactgcctacactggactgttctgagctgagatgagctggggtgagctcagctatgctacgctgtgttggggtgagctgatctgaaatgagatactctggagtagctgagatggggtgagatggggtgagctgagctgggctgagctagactgagctgagctagggtgagctgagctgggtgagctgagctaagctggggtgagctgagctgagcttggctgagctagggtgagctgggctgagctggggtgagctgagctgagctggggtaagctgggatgagctggggtgagctgagctgagctggagtgagctgagctgggctgagctggggtgagctgggctgagctgggctgagctgggctgagctggggtgagctgagctggggtgagctgagctgagctggggtgagctgagctgagctggggtgagctggggtgagctgagctggggtgagctgagctgagctggggtgagctgagctggggtgagctgagctgagctggggtgagctgagctgagctgagctgagctgagctggggtgagctgagctgagctgagctggggtgagctggggtgagctgagctgagctggagtgagctgagctgggctgagctggggtgagctgggctgagctggggtgagctgagctgagctgagctgagctggggtgagctgagctgagctggggtgagctgagctggggtgagctgggctgagctgagctgagctgagctgagctgagctgagctgagctgagctgagctgagctgagctgagctgagctgagctgagctgagctggggtgagctgagctgagctgggctgagctggggtgagctgggctgagctgggctgagctgggctgagctggggtgagctgagctggggtgagctgagctgagctgggctgagctgagctgagctggggtgagctgagctgagctggggtgagctgagctgagctgagctggggtgagctgagctgggctgagcagggctgagctggggtgagctgagctgagctggggtgagctgggctgagctgggctgagctgagctgagctgggctgagctgggctgagctgggctgagctgggctgagctgggctgagctggggtgagctgagctgagctggggtgagctggggtgagctgagctggggtgagctgagctggggtgagctgagctgagctggggtgagctgagctggggtgagctgagctgagctggggtgagctgagctgagctggggtgagctgagctagggtgaactgggctgggtgagctggagtgagctgagctgaggtgaactggggtgagccgggatgttttgagttgagctggggtaagatgagctgaactggggtaaactgggatgagctgtggtgagcggagctggattgaactgagctgtgtgagctgagctggggtcagctgagcaagagtgagtagagctggctggccagaaccagaatcaattaggctaagtgagccagattgtgctgggatcagctgtactcagatgagctgggatgaggtaggctgggatgagctgggctagctgacatggattatgtgaggctgagctagcatgggctggcctagctgatgagctaagcttgaatgagcggggctgagctggactcagatgtgctagactgagctgtactggatgatctggtgtagggtgatctggactcaactgggctggctgatgggatgcgccaggttgaactaggctcagataagttaggctgagtagggcctggttgagatggttcgggatgagctgggaaaagatggactcggaccatgaactgggctgagctgggttgggagaccatgaattgagctgaactgagtgcagctgggataaactgggttgagctaagaatagactacctgaattgtgccaaactcggctgggatcaattggaaattatcaggatttagatgagccggactaaactatgctgagctggactggttggatgtgttgaactggcctgctgctgggctggcatagctgagttgaacttaaatgaggaaggctgagcaaggctagcctgcttgcatagagctgaactttagcctagcctgagctggaccagcctgagctgagtaggtctaaactgagttaaaaatcaacagggataatttaacagctaatttaacaagcctgaggtctgagattgaatgagcagagctgggatgaactgaatgagtttcaccaggcctggaccagttaggctaggacctcgttctatagaggcagactgtgtgctacagtggagtttcaagatgattccatgagtcctccccgcccccaacataacccaccttcctcctaccctacacgcctgtctggtgtgtaaatcccagctttgtgtgctgatacagaagcctgagcccctcccccacctccacctacctattactttgggatgagaatagttctcccagccagtgtctcagagggaagccaagcaggacaggcccaaggctacttgagaagccaggatctaggcctctccctgagaacgggtgttcatgcccctagagttggctgaagggccagatccacctactctagaggcatctctccctgtctgtgaaggcttccaaagtcacgttcctgtggctagaaggcagctccatagccctgctgcagtttcgtcctgtataccaggttcacctactaccatatctagccctgcctgccttaagagtagcaacaaggaaatagcagggtgtagagggatctcctgtctgacaggaggcaagaagacagattcttacccctccatttctcttttatccctctctggtcctcagagagtcagtccttcccaaatgtcttcccccgaaaaccaggggagtagaagttcacaagtgattagtctaaggccttagcctagctagaccagccaggatcagcagccatcaccaggaaagggaacttagcccagaagagaaggagatactgcctctgactccctcttgaaaacttctaactatgaccacctaccctcaaggtcatgatcctctaggatagatgtccttgtcatttccaggatcatcctgacctaagcccatacccagggacaaagtctccaagccctgtttggtgccttttctccttcaaactcgagtaacccccagccttctctctgcagagcccagagtgcccataacacagaacccctgtcctccactcaaagagtgtcccccatgcgcaggtaagtcactagaccagagctccactccagggagaatggtaagtgctataaatatccctgcactagaggataagccatttacagatccatttccatctctcttcatcagctccagacctcttgggtggaccatccgtcttcatcttccctccaaagatcaaggatgtactcatgatctccctgagccccatggtcacatgtgtggtggt

SEQ ID NO: 79 - protein, 146 aa, synthetic construct
OVOLOOSGAELARPGASVKLSCKASGYTFTSYGISWKORTGOGLEWGEIYPRSGNTYYNEKFKGKATLTADKSSSTAYMELRSLTSEDSAVYFCARRNWDRGYFDYWGOGTTLTVSSAVAEMNPNVNVFVPPRDGFSGPAPRKSKL

SEQ ID NO: 80 - protein, 162 aa, synthetic construct
QIQLVQSGPELKKPGETVKISCKASGYTFTTYGMSWVKQAPGKGLKWMGWINTYSGVPTYADDFKGRFAFSLETSASTAYLQINNLKNEDTATYFCARSGGNLPYAMDYWGQGTSVTVSSGPPPPCPPCPPSCHPSLSLQRPALEDLLLGSDASLTCTLNGL

SEQ ID NO: 81 - protein, 163 aa, synthetic construct
EVQLQQSGPELVKPGASVKISCKASGYTFTDYYMNWVKQSHGKSLEWIGDINPNNGGTSYNQKFKGKATLTVDKSSSTAYMELRSLTSEDSAVYYCARGITTVVEYYFDYWGQGTTLTVSSGPPPPCPPCPPSCHPSLSLQRPALEDLLLGSDASLTCTLNGL

SEQ ID NO: 82 - protein, 165 aa, synthetic construct
QVQLQQSGPELVKPGASVKISCKASGYTFTDYYINWVKQRPGQGLEWIGWIFPGSGSTYYNEKFKGKATLTVDKSSSTAYMLLSSLTSEDSAVYFCARLLYDYDSSPWYFDYWGQGTTLTVSSGPPPPCPPCPPSCHPSLSLQRPALEDLLLGSDASLTCTLNGL

SEQ ID NO: 83 - protein, 160 aa, synthetic construct
QVQLQQPGTELVKPGASVKLSCKASGYTFTSYWMHWVKQRPGQGLEWIGNINPSNGGTNYNEKFKSKATLTVDKSSSTAYMQLSSLTSEDSAVYYCARGWEEGLFDYWGQGTTLTVSSGPPPPCPPCPPSCHPSLSLQRPALEDLLLGSDASLTCTLNGL